European Patent Application EP 4 317 418 A1, published February 7, 2024. Title: METHOD OF PRODUCING OVARIAN SOMATIC CELL-LIKE CELLS. Applicant: KYOTO UNIVERSITY KYUSHU UNIVERSITY, NATIONAL UNIVERSITY CORPORATION. The sequence listing filed with the application follows.

SEQUENCE LISTING (146 sequences)

SEQ ID NO: 1 - DNA, 20 bp, Artificial sequence
  Synthesized nucleotides
cactcactctccgcagtcag

SEQ ID NO: 2 - DNA, 20 bp, Artificial sequence
  Synthesized nucleotides
gcgcctctcccagaagtatt

SEQ ID NO: 3 - DNA, 22 bp, Artificial sequence
  Synthesized nucleotides
atttataggccagggcatgtgt

SEQ ID NO: 4 - DNA, 22 bp, Artificial sequence
  Synthesized nucleotides
tgttagacaagattcacccccg

SEQ ID NO: 5 - DNA, 22 bp, Artificial sequence
  Synthesized nucleotides
cctctttctcagcagagctgta

SEQ ID NO: 6 - DNA, 22 bp, Artificial sequence
  Synthesized nucleotides
ctctgctacagccagtaggatt

SEQ ID NO: 7 - DNA, 20 bp, Artificial sequence
  Synthesized nucleotides
taacatgaaagcgggacgga

SEQ ID NO: 8 - DNA, 21 bp, Artificial sequence
  Synthesized nucleotides
aggtcatgaaggacactctgc

SEQ ID NO: 9 - DNA, 22 bp, Artificial sequence
  Synthesized nucleotides
aaatgtccccggatctttcgat

SEQ ID NO: 10 - DNA, 22 bp, Artificial sequence
  Synthesized nucleotides
aaaacaaaaagcagggaggacg

SEQ ID NO: 11 - DNA, 22 bp, Artificial sequence
  Synthesized nucleotides
tcccctcagtttatgtcctcct

SEQ ID NO: 12 - DNA, 22 bp, Artificial sequence
  Synthesized nucleotides
gaaagagacgagcccagtagaa

SEQ ID NO: 13 - DNA, 22 bp, Artificial sequence
  Synthesized nucleotides
gagcaaacacacgtattggtcc

SEQ ID NO: 14 - DNA, 20 bp, Artificial sequence
  Synthesized nucleotides
gtgcagtccatggctagacg

SEQ ID NO: 15 - DNA, 20 bp, Artificial sequence
  Synthesized nucleotides
tggccccacaacacagattt

SEQ ID NO: 16 - DNA, 20 bp, Artificial sequence
  Synthesized nucleotides
ggcattgccacaagctgaaa

SEQ ID NO: 17 - DNA, 22 bp, Artificial sequence
  Synthesized nucleotides
ggatgccaagaagtttaaggaa

SEQ ID NO: 18 - DNA, 22 bp, Artificial sequence
  Synthesized nucleotides
gccagtgaaaggaaacaaaact

SEQ ID NO: 19 - DNA, 22 bp, Artificial sequence
  Synthesized nucleotides
tttttccttttgcaacgtgcct

SEQ ID NO: 20 - DNA, 22 bp, Artificial sequence
  Synthesized nucleotides
ggccactggaatcatttctacc

SEQ ID NO: 21 - DNA, 20 bp, Artificial sequence
  Synthesized nucleotides
aacagaagcttcagggctca

SEQ ID NO: 22 - DNA, 20 bp, Artificial sequence
  Synthesized nucleotides
gtgcagtttggtggtgcttt

SEQ ID NO: 23 - DNA, 23 bp, Artificial sequence
  Synthesized nucleotides
catcttctcttggagtgagggag

SEQ ID NO: 24 - DNA, 23 bp, Artificial sequence
  Synthesized nucleotides
agcaatcctcaaactctctagcc

SEQ ID NO: 25 - DNA, 23 bp, Artificial sequence
  Synthesized nucleotides
cagttcccatcataccagcatcc

SEQ ID NO: 26 - DNA, 23 bp, Artificial sequence
  Synthesized nucleotides
agacccagaaagagggaacaatg

SEQ ID NO: 27 - DNA, 22 bp, Artificial sequence
  Synthesized nucleotides
ttgatcatttggtgtgttgggc

SEQ ID NO: 28 - DNA, 22 bp, Artificial sequence
  Synthesized nucleotides
aagactgagatgcacaagtggt

SEQ ID NO: 29 - DNA, 22 bp, Artificial sequence
  Synthesized nucleotides
gaaactctgcattctcgcttcc

SEQ ID NO: 30 - DNA, 22 bp, Artificial sequence
  Synthesized nucleotides
actcgtttgtacccgttgatga

SEQ ID NO: 31 - DNA, 20 bp, Artificial sequence
  Synthesized nucleotides
tccccacaggcacattaact

SEQ ID NO: 32 - DNA, 21 bp, Artificial sequence
  Synthesized nucleotides
tctcacacattcaccacacca

SEQ ID NO: 33 - DNA, 20 bp, Artificial sequence
  Synthesized nucleotides
gcagggtacaggacaacaca

SEQ ID NO: 34 - DNA, 22 bp, Artificial sequence
  Synthesized nucleotides
aggatgtgttaatggggtgact

SEQ ID NO: 35 - DNA, 21 bp, Artificial sequence
  Synthesized nucleotides
tctactggaatgtccccttgc

SEQ ID NO: 36 - DNA, 21 bp, Artificial sequence
  Synthesized nucleotides
tactctctgcttccgttcctc

SEQ ID NO: 37 - DNA, 22 bp, Artificial sequence
  Synthesized nucleotides
cggcaggtcaaaatctggtttc

SEQ ID NO: 38 - DNA, 22 bp, Artificial sequence
  Synthesized nucleotides
gggtttaggactgctccttgtc

SEQ ID NO: 39 - DNA, 20 bp, Artificial sequence
  Synthesized nucleotides
aggactgggaaagcggaaac

SEQ ID NO: 40 - DNA, 21 bp, Artificial sequence
  Synthesized nucleotides
gcagcacgaacataatgaccc

SEQ ID NO: 41 - DNA, 20 bp, Artificial sequence
  Synthesized nucleotides
cgattccttcccacggtcaa

SEQ ID NO: 42 - DNA, 20 bp, Artificial sequence
  Synthesized nucleotides
tattaggatccgctcggcca

SEQ ID NO: 43 - DNA, 23 bp, Artificial sequence
  Synthesized nucleotides
gatcccggaagatacgctctaag

SEQ ID NO: 44 - DNA, 23 bp, Artificial sequence
  Synthesized nucleotides
cgcaggttgatgcttccaataaa

SEQ ID NO: 45 - DNA, 19 bp, Artificial sequence
  Synthesized nucleotides
tggcaatggcctctcacct

SEQ ID NO: 46 - DNA, 21 bp, Artificial sequence
  Synthesized nucleotides
gagagcgcgtaatcagtctgg

SEQ ID NO: 47 - DNA, 20 bp, Artificial sequence
  Synthesized nucleotides
gctaaagccccagagacgtg

SEQ ID NO: 48 - DNA, 19 bp, Artificial sequence
  Synthesized nucleotides
cgccggtaaggttttgctg

SEQ ID NO: 49 - DNA, 20 bp, Artificial sequence
  Synthesized nucleotides
gattcaggattgcggggacg

SEQ ID NO: 50 - DNA, 25 bp, Artificial sequence
  Synthesized nucleotides
gcggtgttttggttattagggaaag

SEQ ID NO: 51 - DNA, 20 bp, Artificial sequence
  Synthesized nucleotides
ttgagcgtccttcctaccct

SEQ ID NO: 52 - DNA, 20 bp, Artificial sequence
  Synthesized nucleotides
ggagtactcgttcccctgtt

SEQ ID NO: 53 - DNA, 19 bp, Artificial sequence
  Synthesized nucleotides
gcagttggcacatagcctc

SEQ ID NO: 54 - DNA, 21 bp, Artificial sequence
  Synthesized nucleotides
ttgttgcgaatctgagccttc

SEQ ID NO: 55 - DNA, 20 bp, Artificial sequence
  Synthesized nucleotides
tggccgagttcaaccattca

SEQ ID NO: 56 - DNA, 20 bp, Artificial sequence
  Synthesized nucleotides
agtgcttgaaaacttgccgc

SEQ ID NO: 57 - DNA, 20 bp, Artificial sequence
  Synthesized nucleotides
gcgcccagtacagaatacac

SEQ ID NO: 58 - DNA, 19 bp, Artificial sequence
  Synthesized nucleotides
aagagtcggggctactcca

SEQ ID NO: 59 - DNA, 23 bp, Artificial sequence
  Synthesized nucleotides
taaaagaaaataggggctggtcc

SEQ ID NO: 60 - DNA, 21 bp, Artificial sequence
  Synthesized nucleotides
cctcacccaggaagtctcatt

SEQ ID NO: 61 - DNA, 29 bp, Artificial sequence
  Synthesized nucleotides
tggctatagcagagaatacctttgaacca

SEQ ID NO: 62 - DNA, 24 bp, Artificial sequence
  Synthesized nucleotides
acaggtttgtgggttagggagggt

SEQ ID NO: 63 - DNA, 21 bp, Artificial sequence
  Synthesized nucleotides
cgctgcagttgtttcccatta

SEQ ID NO: 64 - DNA, 20 bp, Artificial sequence
  Synthesized nucleotides
gtggaggagaaaagaggcgt

SEQ ID NO: 65 - DNA, 20 bp, Artificial sequence
  Synthesized nucleotides
cacccccagcttcataccaa

SEQ ID NO: 66 - DNA, 22 bp, Artificial sequence
  Synthesized nucleotides
tggggctatgtttcagaaggag

SEQ ID NO: 67 - DNA, 19 bp, Artificial sequence
  Synthesized nucleotides
tgaaccgcccctgtaatcg

SEQ ID NO: 68 - DNA, 22 bp, Artificial sequence
  Synthesized nucleotides
gcgaacaaaacgaaggcaatac

SEQ ID NO: 69 - DNA, 21 bp, Artificial sequence
  Synthesized nucleotides
tagtttagtcccctcacccct

SEQ ID NO: 70 - DNA, 18 bp, Artificial sequence
  Synthesized nucleotides
tccgcactgttgtcgctc

SEQ ID NO: 71 - DNA, 22 bp, Artificial sequence
  Synthesized nucleotides
actgtagagcatccatccatcc

SEQ ID NO: 72 - DNA, 21 bp, Artificial sequence
  Synthesized nucleotides
ttcgtggactaaccacacaca

SEQ ID NO: 73 - DNA, 20 bp, Artificial sequence
  Synthesized nucleotides
tcaccccttggtctctttgc

SEQ ID NO: 74 - DNA, 18 bp, Artificial sequence
  Synthesized nucleotides
actcgcgttccagttcgc

SEQ ID NO: 75 - DNA, 20 bp, Artificial sequence
  Synthesized nucleotides
atgtaaccccacctctccac

SEQ ID NO: 76 - DNA, 21 bp, Artificial sequence
  Synthesized nucleotides
atgctctaaccagccatctca

SEQ ID NO: 77 - DNA, 20 bp, Artificial sequence
  Synthesized nucleotides
ctctgccccctgaaatgtgt

SEQ ID NO: 78 - DNA, 20 bp, Artificial sequence
  Synthesized nucleotides
ggggctggggtgattcttaa

SEQ ID NO: 79 - DNA, 21 bp, Artificial sequence
  Synthesized nucleotides
acagatttgcagggcttttgg

SEQ ID NO: 80 - DNA, 24 bp, Artificial sequence
  Synthesized nucleotides
ggcaactgtctgaatagcatgttt

SEQ ID NO: 81 - DNA, 20 bp, Artificial sequence
  Synthesized nucleotides
aatgatccgccttgacaccc

SEQ ID NO: 82 - DNA, 21 bp, Artificial sequence
  Synthesized nucleotides
tcaccttcctgcatctggttc

SEQ ID NO: 83 - DNA, 21 bp, Artificial sequence
  Synthesized nucleotides
gcctgccacttcaatgttcag

SEQ ID NO: 84 - DNA, 22 bp, Artificial sequence
  Synthesized nucleotides
taggagaaagggtacaggcagg

SEQ ID NO: 85 - DNA, 28 bp, Artificial sequence
  Synthesized nucleotides
tcatgtagtttgtataaaatgtgggaag

SEQ ID NO: 86 - DNA, 29 bp, Artificial sequence
  Synthesized nucleotides
aaaacttgtaaatagttggccttacaaaa

SEQ ID NO: 87 - DNA, 20 bp, Artificial sequence
  Synthesized nucleotides
tctggatgctgctaacccac

SEQ ID NO: 88 - DNA, 20 bp, Artificial sequence
  Synthesized nucleotides
gtcacaatggcaaagagcct

SEQ ID NO: 89 - DNA, 21 bp, Artificial sequence
  Synthesized nucleotides
ggcctctaggaggaaaccaac

SEQ ID NO: 90 - DNA, 20 bp, Artificial sequence
  Synthesized nucleotides
actaacctcacccaccatcc

SEQ ID NO: 91 - DNA, 20 bp, Artificial sequence
  Synthesized nucleotides
ggcatgcatcgaggaatcgt

SEQ ID NO: 92 - DNA, 19 bp, Artificial sequence
  Synthesized nucleotides
tgcacagatgccagtggtc

SEQ ID NO: 93 - DNA, 20 bp, Artificial sequence
  Synthesized nucleotides
cgacctaggtggtcttgtgg

SEQ ID NO: 94 - DNA, 22 bp, Artificial sequence
  Synthesized nucleotides
ttggtcccccaaacaagttaca

SEQ ID NO: 95 - DNA, 23 bp, Artificial sequence
  Synthesized nucleotides
gattatagtgtccacttgccacc

SEQ ID NO: 96 - DNA, 24 bp, Artificial sequence
  Synthesized nucleotides
aagggtatatctgtgcatccatct

SEQ ID NO: 97 - DNA, 20 bp, Artificial sequence
  Synthesized nucleotides
ctgatccctcaggtctgctg

SEQ ID NO: 98 - DNA, 21 bp, Artificial sequence
  Synthesized nucleotides
acttcctgggcaaactgttga

SEQ ID NO: 99 - DNA, 25 bp, Artificial sequence
  Synthesized nucleotides
ggttcagtaacattaaggaccatga

SEQ ID NO: 100 - DNA, 25 bp, Artificial sequence
  Synthesized nucleotides
aaagaaaatggacagagaaatgcaa

SEQ ID NO: 101 - DNA, 22 bp, Artificial sequence
  Synthesized nucleotides
agagtaaactgctctgttccca

SEQ ID NO: 102 - DNA, 22 bp, Artificial sequence
  Synthesized nucleotides
tttgacaagcagactgacatcc

SEQ ID NO: 103 - DNA, 22 bp, Artificial sequence
  Synthesized nucleotides
agccaaggaatgtgtccaagac

SEQ ID NO: 104 - DNA, 22 bp, Artificial sequence
  Synthesized nucleotides
aattcaagaactaagcgggacc

SEQ ID NO: 105 - DNA, 23 bp, Artificial sequence
  Synthesized nucleotides
agatgcaattttcctccattcct

SEQ ID NO: 106 - DNA, 27 bp, Artificial sequence
  Synthesized nucleotides
tgtatcagtttgaacctagaagattga

SEQ ID NO: 107 - DNA, 20 bp, Artificial sequence
  Synthesized nucleotides
gagatccttgcctggggaaa

SEQ ID NO: 108 - DNA, 20 bp, Artificial sequence
  Synthesized nucleotides
tgtgacggatgagattccct

SEQ ID NO: 109 - DNA, 23 bp, Artificial sequence
  Synthesized nucleotides
ccgaaaccttcaagataaaggca

SEQ ID NO: 110 - DNA, 20 bp, Artificial sequence
  Synthesized nucleotides
tttgagcgtgacacttctcc

SEQ ID NO: 111 - DNA, 23 bp, Artificial sequence
  Synthesized nucleotides
ggatggggacttgtgaatttttc

SEQ ID NO: 112 - DNA, 19 bp, Artificial sequence
  Synthesized nucleotides
ggtggaaagtgagcaacgg

SEQ ID NO: 113 - DNA, 22 bp, Artificial sequence
  Synthesized nucleotides
gctggcctgagaaacacaattt

SEQ ID NO: 114 - DNA, 24 bp, Artificial sequence
  Synthesized nucleotides
acgtccctcttcacaaaaatagga

SEQ ID NO: 115 - DNA, 20 bp, Artificial sequence
  Synthesized nucleotides
acaacgacgaggagattcgt

SEQ ID NO: 116 - DNA, 20 bp, Artificial sequence
  Synthesized nucleotides
gcttgcagagtcattcacgg

SEQ ID NO: 117 - DNA, 21 bp, Artificial sequence
  Synthesized nucleotides
gctttacggctcaagaatgcc

SEQ ID NO: 118 - DNA, 20 bp, Artificial sequence
  Synthesized nucleotides
tgctgtgcagtgaatgggag

SEQ ID NO: 119 - DNA, 20 bp, Artificial sequence
  Synthesized nucleotides
acccaggagtgatcggagac

SEQ ID NO: 120 - DNA, 21 bp, Artificial sequence
  Synthesized nucleotides
ggacagaggactgaagctgta

SEQ ID NO: 121 - DNA, 20 bp, Artificial sequence
  Synthesized nucleotides
tcatacgccagaggacagac

SEQ ID NO: 122 - DNA, 23 bp, Artificial sequence
  Synthesized nucleotides
cacagtcattcagaatcagccac

SEQ ID NO: 123 - DNA, 20 bp, Artificial sequence
  Synthesized nucleotides
caggctgagggtagcaccta

SEQ ID NO: 124 - DNA, 20 bp, Artificial sequence
  Synthesized nucleotides
gtcgggggttgcatctctaa

SEQ ID NO: 125 - DNA, 20 bp, Artificial sequence
  Synthesized nucleotides
cgtggtcagagtagaacccc

SEQ ID NO: 126 - DNA, 23 bp, Artificial sequence
  Synthesized nucleotides
tccacgaccacatacaatgattc

SEQ ID NO: 127 - DNA, 19 bp, Artificial sequence
  Synthesized nucleotides
ggagccgggcgttatattg

SEQ ID NO: 128 - DNA, 25 bp, Artificial sequence
  Synthesized nucleotides
aactccagtgataaatgtccgttac

SEQ ID NO: 129 - DNA, 24 bp, Artificial sequence
  Synthesized nucleotides
gtggagccatatgaatgtcagtag

SEQ ID NO: 130 - DNA, 23 bp, Artificial sequence
  Synthesized nucleotides
tgtggctaacattgaaaagctgc

SEQ ID NO: 131 - DNA, 23 bp, Artificial sequence
  Synthesized nucleotides
cccacttttctaacttttcgccc

SEQ ID NO: 132 - DNA, 22 bp, Artificial sequence
  Synthesized nucleotides
aaaagcaagttgatgggtcagc

SEQ ID NO: 133 - DNA, 22 bp, Artificial sequence
  Synthesized nucleotides
attccagtatccccaaagcctg

SEQ ID NO: 134 - DNA, 21 bp, Artificial sequence
  Synthesized nucleotides
gatctcagcgacacccacatc

SEQ ID NO: 135 - DNA, 20 bp, Artificial sequence
  Synthesized nucleotides
aacagggtggtggacctcat

SEQ ID NO: 136 - DNA, 20 bp, Artificial sequence
  Synthesized nucleotides
ttcctcttgtgctctcgctg

SEQ ID NO: 137 - DNA, 20 bp, Artificial sequence
  Synthesized nucleotides
acaggtcctggcatcttgtc

SEQ ID NO: 138 - DNA, 20 bp, Artificial sequence
  Synthesized nucleotides
ctcagtcttggcagtgcaga

SEQ ID NO: 139 - DNA, 23 bp, Artificial sequence
  Synthesized nucleotides
gatcccggaagatacgctctaag

SEQ ID NO: 140 - DNA, 23 bp, Artificial sequence
  Synthesized nucleotides
cgcaggttgatgcttccaataaa

SEQ ID NO: 141 - DNA, 22 bp, Artificial sequence
  Synthesized nucleotides
aattacagttaggccgctgaca

SEQ ID NO: 142 - DNA, 22 bp, Artificial sequence
  Synthesized nucleotides
ataagcgctgtcacggatgtat

SEQ ID NO: 143 - DNA, 22 bp, Artificial sequence
  Synthesized nucleotides
atcacttctggccgtccttatg

SEQ ID NO: 144 - DNA, 22 bp, Artificial sequence
  Synthesized nucleotides
ttccccaatgaccttaactccg

SEQ ID NO: 145 - DNA, 22 bp, Artificial sequence
  Synthesized nucleotides
ctacccagataacatcgctccc

SEQ ID NO: 146 - DNA, 22 bp, Artificial sequence
  Synthesized nucleotides
tatcagtacttccaagcagccc